European Patent Application EP 4 512 419 A1, published February 26, 2025. Title: POLYVALENT PNEUMOCOCCAL POLYSACCHARIDE CONJUGATE VACCINE COMPONENT AND APPLICATION THEREOF. Applicant: SHANGHAI REINOVAX BIOLOGICS CO., LTD. The sequence listing filed with the application follows.

SEQUENCE LISTING (3 sequences)

SEQ ID NO: 1 - DNA, 1353 bp, synthetic construct
  misc_feature 1..1353: note = TTD
  source 1..1353: mol_type = other DNA
aaaaaccttgactgctgggtggataacgaagaggacatcgacgtcatattgaaaaaatcgactattttaaatttagacattaacaatgacattatttcggacatttcaggctttaactcatcagtaataacttatcctgacgcacaattggtccctggaatcaacggtaaagccatccatctggtgaacaacgaaagttccgaagtgattgtccataaagctatggacattgagtataacgatatgtttaataatttcactgtgagtttttggctgcgtgtccctaaagtatctgccagtcacttagagcaatatggtacgaacgaatactcgataatttcatctatgaaaaaacatagcttgtcaatcggctcaggctggtccgtctcactgaagggcaataatcttatctggaccctgaaggactctgcgggtgaagtacggcagatcacgtttagagatcttccggataaatttaacgcttatttagcgaacaaatgggtctttatcactatcacaaatgatcgtctgtcgagcgccaacctttatattaacggagtactgatgggtagtgctgagattaccggacttggagcgattcgggaagacaacaacatcacccttaaacttgatcgttgtaacaataataatcagtacgtgagcatcgacaagtttcggatattttgtaaggcgttaaatccgaaggaaattgaaaaattatatacatcgtatctgtcaatcactttcttgcgggatttctgggggaatcctcttcggtatgataccgaatactatcttatacctgtggcatctagtagtaaggatgtacagttgaagaacattacagattatatgtatcttaccaatgcacccagttacacaaacggcaagttaaatatctattatcgccggctttataacggtctgaaattcatcataaaaagatacactcccaacaacgagatagattcttttgtcaagagcggagacttcattaagttatatgtcagctacaacaacaatgagcacatagttggctacccaaaggacggaaacgcgtttaacaacctggatcgtatactgcgggtgggctataacgcgcctgggattcccttgtataaaaagatggaagcagtaaaattgcgcgacttgaagacgtactccgtacaacttaaactttacgacgacaaaaatgcgagtcttggattggttggtacgcacaacggacagatcgggaatgatccgaaccgtgacatcttaattgcatcaaattggtactttaatcatttgaaagacaaaatccttggctgcgattggtattttgttccgactgatgaggggtggacgaacgac

SEQ ID NO: 2 - protein, 451 aa, synthetic construct
  REGION 1..451: note = TTD
KNLDCWVDNEEDIDVILKKSTILNLDINNDIISDISGFNSSVITYPDAQLVPGINGKAIHLVNNESSEVIVHKAMDIEYNDMFNNFTVSFWLRVPKVSASHLEQYGTNEYSIISSMKKHSLSIGSGWSVSLKGNNLIWTLKDSAGEVRQITFRDLPDKFNAYLANKWVFITITNDRLSSANLYINGVLMGSAEITGLGAIREDNNITLKLDRCNNNNQYVSIDKFRIFCKALNPKEIEKLYTSYLSITFLRDFWGNPLRYDTEYYLIPVASSSKDVQLKNITDYMYLTNAPSYTNGKLNIYYRRLYNGLKFIIKRYTPNNEIDSFVKSGDFIKLYVSYNNNEHIVGYPKDGNAFNNLDRILRVGYNAPGIPLYKKMEAVKLRDLKTYSVQLKLYDDKNASLGLVGTHNGQIGNDPNRDILIASNWYFNHLKDKILGCDWYFVPTDEGWTND

SEQ ID NO: 3 - protein, 536 aa, synthetic construct
  REGION 1..536: note = CRM197
MGADDVVDSSKSFVMENFSSYHGTKPGYVDSIQKGIQKPKSGTQGNYDDDWKEFYSTDNKYDAAGYSVDNENPLSGKAGGVVKVTYPGLTKVLALKVDNAETIKKELGLSLTEPLMEQVGTEEFIKRFGDGASRVVLSLPFAEGSSSVEYINNWEQAKALSVELEINFETRGKRGQDAMYEYMAQACAGNRVRRSVGSSLSCINLDWDVIRDKTKTKIESLKEHGPIKNKMSESPNKTVSEEKAKQYLEEFHQTALEHPELSELKTVTGTNPVFAGANYAAWAVNVAQVIDSETADNLEKTTAALSILPGIGSVMGIADGAVHHNTEEIVAQSIALSSLMVAQAIPLVGELVDIGFAAYNFVESIINLFQVVHNSYNRPAYSPGHKTQPFLHDGYAVSWNTVEDSIIRTGFQGESGHDIKITAENTPLPIAGVLLPTIPGKLDVNKSKTHISVNGRKIRMRCRAIDGDVTFCRPKSPVYVGNGVHANLHVAFHRSSSEKIHSNEISSDSIGVLGYQKTVDHTKVNSKLSLFFEIKS